European Patent Specification EP 3 639 845 B1, published June 21, 2023. Title: IL-15 PROTEIN COMPLEX PHARMACEUTICAL COMPOSITION AND USES THEREOF. Applicant: JIANGSU HENGRUI MEDICINE CO.,LTD; SHANGHAI HENGRUI PHARMACEUTICAL CO.,LTD. The sequence listing filed with the application follows.

SEQUENCE LISTING (2 sequences)

SEQ ID NO: 1 - protein, 114 aa, artificial sequence
  IL-15 (L52C)
NWVNVISDLKKIEDLIQSMHIDATLYTESDVHPSCKVTAMKCFLLELQVISCESGDASIHDTVENLIILANNSLSSNGNVTESGCKECEELEEKNIKEFLQSFVHIVQMFINTS

SEQ ID NO: 2 - protein, 315 aa, artificial sequence
  IL-15R alpha-Sushi+(S40C)-Fc
ITCPPPMSVEHADIWVKSYSLYSRERYICNSGFKRKAGTCSLTECVLNKATNVAHWTTPSLKCIRDPALVHQRGGGGSGGGGSEPKSSDKTHTCPPCPAPELLGGPSVFLFPPKPKDTLMISRTPEVTCVVVDVSHEDPEVKFNWYVDGVEVHNAKTKPREEQYNSTYRVVSVLTVLHQDWLNGKEYKCKVSNKALPAPIEKTISKAKGQPREPQVYTLPPSREEMTKNQVSLTCLVKGFYPSDIAVEWESNGQPENNYKTTPPVLDSDGSFFLYSKLTVDKSRWQQGNVFSCSVMHEALHNHYTQKSLSLSPGK